European Patent Application EP 4 573 907 A1, published June 25, 2025. Title: Acide butyrique, sel d'acide butyrique ou dérivé d'acide butyrique pour la stimulation et/ou désinhibition des réponses immunitaire des plantes et/ou le traitement d'infections de plantes. Applicant: Université de Bourgogne. The sequence listing filed with the application follows.

SEQUENCE LISTING (10 sequences)

SEQ ID NO: 1 - DNA, 21 bp, synthetic construct
  source 1..21: mol_type = other DNA; note = STS amorce sens
aggaagcagcattgaaggctc

SEQ ID NO: 2 - DNA, 21 bp, synthetic construct
  source 1..21: mol_type = other DNA; note = STS amorce antisens
tgcaccaggcatttctacacc

SEQ ID NO: 3 - DNA, 21 bp, synthetic construct
  source 1..21: mol_type = other DNA; note = PAL amorce sens
agtctccatggacaacacccg

SEQ ID NO: 4 - DNA, 21 bp, synthetic construct
  source 1..21: mol_type = other DNA; note = PAL amorce antisens
tgctcagcactttcgacatgg

SEQ ID NO: 5 - DNA, 21 bp, synthetic construct
  source 1..21: mol_type = other DNA; note = PR3 amorce sens
gcaaccgatgttgacatatca

SEQ ID NO: 6 - DNA, 19 bp, synthetic construct
  source 1..19: mol_type = other DNA; note = PR3 amorce antisens
cgtcgccctagcaagtgag

SEQ ID NO: 7 - DNA, 20 bp, synthetic construct
  source 1..20: mol_type = other DNA; note = VATP16 amorce sens
cttctcctgtatgggagctg

SEQ ID NO: 8 - DNA, 23 bp, synthetic construct
  source 1..23: mol_type = other DNA; note = VATP16 amorce antisens
ccataacaactggtacaatcgac

SEQ ID NO: 9 - DNA, 20 bp, synthetic construct
  source 1..20: mol_type = other DNA; note = EF1-alpha amorce sens
tctgccttcttccttgggta

SEQ ID NO: 10 - DNA, 20 bp, synthetic construct
  source 1..20: mol_type = other DNA; note = EF1-alpha amorce antisens
gcacttcgatcaaaagagga